European Patent Application EP 4 763 985 A1, published June 24, 2026. Title: ANTISENSE OLIGONUCLEOTIDES AS THERAPEUTIC AGENTS AGAINST SARS CoV-2. Applicant: CENTRE NATIONAL DE LA RECHERCHE SCIENTIFIQUE. The sequence listing filed with the application follows.

SEQUENCE LISTING (49 sequences)

SEQ ID NO: 1 - RNA, 21 nt, synthetic construct
  source 1..21: mol_type = other RNA
  misc_difference 5: note = t or u
  misc_difference 17: note = t or u
  misc_difference 19: note = t or u
cccgtttaaaaacgattgtgc

SEQ ID NO: 2 - RNA, 21 nt, synthetic construct
  source 1..21: mol_type = other RNA
  misc_difference 1: note = t or u
  misc_difference 21: note = t or u
tcacaactacagccataacct

SEQ ID NO: 3 - RNA, 21 nt, synthetic construct
  source 1..21: mol_type = other RNA
  misc_difference 2: note = t or u
gtcaaaagccctgtatacgac

SEQ ID NO: 4 - RNA, 21 nt, synthetic construct
  source 1..21: mol_type = other RNA
  misc_difference 19: note = t or u
gcacggtgtaagacgggctgc

SEQ ID NO: 5 - RNA, 20 nt, synthetic construct
  source 1..20: mol_type = other RNA
  misc_difference 17: note = t or u
cggagttgatcacaactaca

SEQ ID NO: 6 - RNA, 21 nt, synthetic construct
  source 1..21: mol_type = other RNA
ccgcaaacccgtttaaaaacg

SEQ ID NO: 7 - RNA, 21 nt, synthetic construct
  source 1..21: mol_type = other RNA
cgtttttaaacgggtttgcgg

SEQ ID NO: 8 - RNA, 21 nt, synthetic construct
  source 1..21: mol_type = other RNA
gcacaatcgtttttaaacggg

SEQ ID NO: 9 - RNA, 21 nt, synthetic construct
  source 1..21: mol_type = other RNA
gcagcccgtcttacaccgtgc

SEQ ID NO: 10 - RNA, 21 nt, synthetic construct
  source 1..21: mol_type = other RNA
gtcgtatacagggcttttgac

SEQ ID NO: 11 - DNA, 37 bp, synthetic construct
  source 1..37: mol_type = other DNA
gaaaaacacgatgataatatggcttccaaggtgtacg

SEQ ID NO: 12 - DNA, 40 bp, synthetic construct
  source 1..40: mol_type = other DNA
caccgcaaacccgtttaaaaactgctcgttcttcagcacg

SEQ ID NO: 13 - DNA, 54 bp, synthetic construct
  source 1..54: mol_type = other DNA
tttttaaacgggtttgcggtgtaagtgcagcccgtcttacaccgtgcggcacag

SEQ ID NO: 14 - DNA, 56 bp, synthetic construct
  source 1..56: mol_type = other DNA
gtcaaaagccctgtatacgacatcagtactagtgcctgtgccgcacggtgtaagac

SEQ ID NO: 15 - DNA, 49 bp, synthetic construct
  source 1..49: mol_type = other DNA
gtcgtatacagggcttttgacatggaagatgccaaaaacattaagaagg

SEQ ID NO: 16 - DNA, 42 bp, synthetic construct
  source 1..42: mol_type = other DNA
gcgtcgacgagctcctgcagttattacacggcgatcttgccg

SEQ ID NO: 17 - DNA, 34 bp, synthetic construct
  source 1..34: mol_type = other DNA
catattatcatcgtgtttttcaaaggaaaaccac

SEQ ID NO: 18 - DNA, 44 bp, synthetic construct
  source 1..44: mol_type = other DNA
ggctggtgctggggtcggtgctcatctgctcgttcttcagcacg

SEQ ID NO: 19 - DNA, 44 bp, synthetic construct; identical to SEQ ID NO: 18
  source 1..44: mol_type = other DNA

SEQ ID NO: 20 - DNA, 53 bp, synthetic construct
  source 1..53: mol_type = other DNA
caccgaccccagcaccagcctgagcatggaagatgccaaaaacattaagaagg

SEQ ID NO: 21 - DNA, 39 bp, synthetic construct
  source 1..39: mol_type = other DNA
ttggcatcttccatggatccctgctcgttcttcagcacg

SEQ ID NO: 22 - DNA, 48 bp, synthetic construct
  source 1..48: mol_type = other DNA
tgaagaacgagcagggatccatggaagatgccaaaaacattaagaagg

SEQ ID NO: 23 - DNA, 47 bp, synthetic construct
  source 1..47: mol_type = other DNA
agcgcgtgctgaagaacgagcaggaattcacagtctgtaccgtctgc

SEQ ID NO: 24 - DNA, 28 bp, synthetic construct
  source 1..28: mol_type = other DNA
ccttcttaatgtttttggcatcttccat

SEQ ID NO: 25 - DNA, 22 bp, synthetic construct
  source 1..22: mol_type = other DNA
taatcagacaaggaactgatta

SEQ ID NO: 26 - DNA, 19 bp, synthetic construct
  source 1..19: mol_type = other DNA
cgaaggtgtgacttccatg

SEQ ID NO: 27 - RNA, 21 nt, synthetic construct
  source 1..21: mol_type = other RNA
attgtagatgtcaaaatgcac

SEQ ID NO: 28 - RNA, 21 nt, synthetic construct
  source 1..21: mol_type = other RNA
cagtactagtgcctgtgccgc

SEQ ID NO: 29 - RNA, 21 nt, synthetic construct
  source 1..21: mol_type = other RNA
ccgtttaaaaacgattgtgca

SEQ ID NO: 30 - RNA, 21 nt, synthetic construct
  source 1..21: mol_type = other RNA
cccgtttaaaaacgattgtgc

SEQ ID NO: 31 - RNA, 21 nt, synthetic construct
  source 1..21: mol_type = other RNA
  misc_difference 1..5: note = 2'-O-methyl base
  misc_difference 17..21: note = 2'-O-methyl base
  misc_difference 1..21: note = phosphorothioate bonds
ccgcaaacccgtttaaaaacg

SEQ ID NO: 32 - RNA, 21 nt, synthetic construct
  source 1..21: mol_type = other RNA
  misc_difference 1..2: note = 2'-O-methoxyethyl base
  misc_difference 20..21: note = 2'-O-methoxyethyl base
  misc_difference 3..5: note = 2'-O-methyl base
  misc_difference 17..19: note = 2'-O-methyl base
  misc_difference 1..21: note = phosphorothioate bonds
ccgcaaacccgtttaaaaacg

SEQ ID NO: 33 - RNA, 21 nt, synthetic construct
  source 1..21: mol_type = other RNA
  misc_difference 1..3: note = 2'-O-methoxyethyl base
  misc_difference 21: note = 2'-O-methoxyethyl base
  misc_difference 4..5: note = 2'-O-methyl base
  misc_difference 17..20: note = 2'-O-methyl base
  misc_difference 1..21: note = phophorothioate bonds
cccgtttaaaaacgattgtgc

SEQ ID NO: 34 - RNA, 21 nt, synthetic construct
  source 1..21: mol_type = other RNA
  misc_difference 1..3: note = 2'-O-methoxyethyl base
  misc_difference 21: note = 2'-O-methoxyethyl base
  misc_difference 4..5: note = 2'-O-methyl base
  misc_difference 17..20: note = 2'-O-methyl base
  misc_difference 1..21: note = phosphorothioate bonds
  misc_difference 1: note = Cyanine (Cy3)
cccgtttaaaaacgattgtgc

SEQ ID NO: 35 - RNA, 21 nt, synthetic construct
  source 1..21: mol_type = other RNA
  misc_difference 1..5: note = 2'-O-methyl base
  misc_difference 17..21: note = 2'-O-methyl base
  misc_difference 1..21: note = phosphorothioate bonds
gcacggtgtaagacgggctgc

SEQ ID NO: 36 - RNA, 21 nt, synthetic construct
  source 1..21: mol_type = other RNA
  misc_difference 1..5: note = 2'-O-methyl base
  misc_difference 17..20: note = 2'-O-methyl base
  misc_difference 21: note = 2'-O-methoxyethyl base
  misc_difference 1..21: note = phosphorothioate bonds
gtcaaaagccctgtatacgac

SEQ ID NO: 37 - RNA, 21 nt, synthetic construct
  source 1..21: mol_type = other RNA
  misc_difference 1: note = 2'-O-methoxyethyl base
  misc_difference 21: note = 2'-O-methoxyethyl base
  misc_difference 2..5: note = 2'-O-methyl base
  misc_difference 17..20: note = 2'-O-methyl base
  misc_difference 1..21: note = phosphorothioate bonds
cggagttgatcacaactacag

SEQ ID NO: 38 - RNA, 21 nt, synthetic construct
  source 1..21: mol_type = other RNA
  misc_difference 1..5: note = 2'-O-methyl base
  misc_difference 17..21: note = 2'-O-methyl base
  misc_difference 1..21: note = phosphorothioate bonds
tcacaactacagccataacct

SEQ ID NO: 39 - RNA, 20 nt, synthetic construct
  source 1..20: mol_type = other RNA
  misc_difference 1..5: note = 2'-O-methyl base
  misc_difference 16..20: note = 2'-O-methyl base
  misc_difference 1..20: note = phosphorothioate bonds
cccacagggtcattagcaca

SEQ ID NO: 40 - RNA, 21 nt, synthetic construct
  source 1..21: mol_type = other RNA
  misc_difference 1..5: note = 2'-O-methyl base
  misc_difference 17..21: note = 2'-O-methyl base
  misc_difference 1..21: note = phosphorothioate bonds
cgtccttttcttggaagcgac

SEQ ID NO: 41 - RNA, 21 nt, synthetic construct
  source 1..21: mol_type = other RNA
  misc_difference 1..3: note = 2'-O-methoxyethyl base
  misc_difference 21: note = 2'-O-methoxyethyl base
  misc_difference 4..5: phenotype = 2'-methyl base
  misc_difference 17..20: note = 2'-O-methyl base
  misc_difference 1..21: note = phosphorothioate bonds
aggaatttagcaaaaccagct

SEQ ID NO: 42 - RNA, 21 nt, synthetic construct
  source 1..21: mol_type = other RNA
  misc_difference 1..2: note = 2'-O-methoxyethyl base
  misc_difference 20..21: note = 2'-O-methoxyethyl base
  misc_difference 3..5: note = 2'-O-methyl base
  misc_difference 17..19: note = 2'-O-methyl base
  misc_difference 1..21: note = phosphorothioate bonds
tactccaatcggaacaacgca

SEQ ID NO: 43 - RNA, 21 nt, synthetic construct
  source 1..21: mol_type = other RNA
  misc_difference 1..2: note = 2'-O-methoxyethyl base
  misc_difference 20..21: note = 2'-O-methoxyethyl base
  misc_difference 3..5: note = 2'-O-methyl base
  misc_difference 17..19: note = 2'-O-methyl base
  misc_difference 1: note = Cyanine (Cy3)
tactccaatcggaacaacgca

SEQ ID NO: 44 - RNA, 189 nt, synthetic construct
  source 1..189: mol_type = other RNA
acagtctgtaccgtctgcggtatgtggaaaggttatggctgtagttgtgatcaactccgcgaacccatgcttcagtcagctgatgcacaatcgtttttaaacgggtttgcggtgtaagtgcagcccgtcttacaccgtgcggcacaggcactagtactgatgtcgtatacagggcttttgacatctaca

SEQ ID NO: 45 - RNA, 151 nt, synthetic construct
  source 1..151: mol_type = other RNA
tggctgtagttgtgatcaactccgcgaacccatgcttcagtcagctgatgcacaatcgtttttaaacgggtttgcggtgtaagtgcagcccgtcttacaccgtgcggcacaggcactagtactgatgtcgtatacagggcttttgacatct

SEQ ID NO: 46 - RNA, 10 nt, synthetic construct
  source 1..10: mol_type = other RNA
agtgcctgcc

SEQ ID NO: 47 - RNA, 189 nt, synthetic construct; identical to SEQ ID NO: 44
  source 1..189: mol_type = other RNA

SEQ ID NO: 48 - RNA, 123 nt, synthetic construct
  source 1..123: mol_type = other RNA
cccatgcttcagtcagctgatgcacaatcgtttttaaacgggtttgcggtgtaagtgcagcccgtcttacaccgtgcggcacaggcactagtactgatgtcgtatacagggcttttgacatct

SEQ ID NO: 49 - RNA, 28 nt, synthetic construct
  source 1..28: mol_type = other RNA
cccatgcttcagtcagctgatgcacaat